European Patent Application EP 4 752 228 A2, published June 3, 2026. Title: DNA Binding Proteins for Regulating Gene Expression. Applicant: Altius Institute for Biomedical Sciences. Application EP. The sequence listing filed with the application follows.

SEQUENCE LISTING (221 sequences)

SEQ ID NO: 1 - protein, 33 aa, synthetic construct
  VARIANT 12: note = The amino acid at position 12 may be His, Lys, Asn, Arg, Ser, Tyr or Cys
  VARIANT 13: note = The amino acid at position 13 may be His, Lys, Gln, Asn, Ile, Gly, Asp, Val, Ala, Ser, or absent
LTPDQVVAIASXXGGKQALETVQRLLPVLQDHG

SEQ ID NO: 2 - protein, 110 aa, Xanthomonas sp.
HHEALVGHGFTHAHIVALSQHPAALGTVAVKYQDMIAALPEATHEAIVGVGKQWSGARALEALLTVAGELRGPPLQLDTGQLLKIAKRGGVTAVEAVHAWRNALTGAPLN

SEQ ID NO: 3 - DNA, 30 bp, Homo sapiens
  source 1..30: mol_type = genomic DNA
agcagtatcctcttgggggccccttcccca

SEQ ID NO: 4-5 - skipped (2 entries)

SEQ ID NO: 6 - protein, 11 aa, Xanthomonas sp.
LTPEQVVAIAS

SEQ ID NO: 7 - protein, 7 aa, synthetic construct
GGRPALE

SEQ ID NO: 8 - DNA, 35 bp, Homo sapiens
  source 1..35: mol_type = genomic DNA
taagcagcagtatcctcttgggggccccttcccca

SEQ ID NO: 9 - protein, 11 aa, Xanthomonas sp.
LTPAQVVAIAS

SEQ ID NO: 10 - protein, 11 aa, Xanthomonas sp.
LTPDQVVAIAN

SEQ ID NO: 11 - protein, 11 aa, Xanthomonas sp.
LTPDQVVAIAS

SEQ ID NO: 12 - protein, 11 aa, Xanthomonas sp.
LTPYQVVAIAS

SEQ ID NO: 13 - protein, 11 aa, Xanthomonas sp.
LTREQVVAIAS

SEQ ID NO: 14 - protein, 11 aa, Xanthomonas sp.
LSTAQVVAIAS

SEQ ID NO: 15 - protein, 21 aa, synthetic construct
GGKQALETVQRLLPVLCQDHG

SEQ ID NO: 16 - protein, 21 aa, synthetic construct
GGKQALATVQRLLPVLCQDHG

SEQ ID NO: 17 - protein, 21 aa, synthetic construct
GGKQALETVQRVLPVLCQDHG

SEQ ID NO: 18 - protein, 120 aa, Xanthomonas sp.
KPKVRSTVAQHHEALVGHGFTHAHIVALSQHPAALGTVAVKYQDMIAALPEATHEAIVGVGKQWSGARALEALLTVAGELRGPPLQLDTGQLLKIAKRGGVTAVEAVHAWRNALTGAPLN

SEQ ID NO: 19 - protein, 115 aa, Xanthomonas sp.
STVAQHHEALVGHGFTHAHIVALSQHPAALGTVAVKYQDMIAALPEATHEAIVGVGKQWSGARALEALLTVAGELRGPPLQLDTGQLLKIAKRGGVTAVEAVHAWRNALTGAPLN

SEQ ID NO: 20 - protein, 110 aa, Xanthomonas sp.; identical to SEQ ID NO: 2

SEQ ID NO: 21 - protein, 34 aa, Xanthomonas sp.
LTPDQVVAIASNHGGKQALETVQRLLPVLCQDHG

SEQ ID NO: 22 - protein, 34 aa, Xanthomonas sp.
LTPDQVVAIASNGGGKQALETVQRLLPVLCQDHG

SEQ ID NO: 23 - protein, 34 aa, Xanthomonas sp.
LTPDQVVAIASNIGGKQALETVQRLLPVLCQDHG

SEQ ID NO: 24 - protein, 34 aa, Xanthomonas sp.
LTPDQVVAIASHDGGKQALETVQRLLPVLCQDHG

SEQ ID NO: 25 - DNA, 19 bp, unidentified
  misc_feature 1..19: note = nucleic acid sequence targeted by a recombinant DNA binding protein (DBP)
  source 1..19: mol_type = other DNA
cttgggggccccttcccca

SEQ ID NO: 26 - protein, 35 aa, Ralstonia solanacearum
LDTEQVVAIASHNGGKQALEAVKADLLDLLGAPYV

SEQ ID NO: 27 - protein, 35 aa, Ralstonia solanacearum
LNTEQVVAVASNKGGKQALEAVGAQLLALRAVPYE

SEQ ID NO: 28 - protein, 35 aa, Ralstonia solanacearum
LSTAQVAAIASHDGGKQALEAVGTQLVVLRAAPYA

SEQ ID NO: 29 - protein, 35 aa, Ralstonia solanacearum
LSTAQVVAVAGRNGGKQALEAVRAQLPALRAAPYG

SEQ ID NO: 30 - protein, 35 aa, Ralstonia solanacearum
LSTAQVVAVASSNGGKQALEAVWALLPVLRATPYD

SEQ ID NO: 31 - protein, 137 aa, Ralstonia solanacearum
FGKLVALGYSREQIRKLKQESLSEIAKYHTTLTGQGFTHADICRISRRRQSLRVVARNYPELAAALPELTRAHIVDIARQRSGDLALQALLPVATALTAAPLRLSASQIATVAQYGERPAIQALYRLRRKLTRAPLH

SEQ ID NO: 32 - protein, 120 aa, Ralstonia solanacearum
KQESLSEIAKYHTTLTGQGFTHADICRISRRRQSLRVVARNYPELAAALPELTRAHIVDIARQRSGDLALQALLPVATALTAAPLRLSASQIATVAQYGERPAIQALYRLRRKLTRAPLH

SEQ ID NO: 33 - protein, 19 aa, Ralstonia solanacearum
LSTAQVVAIACISGQQALE

SEQ ID NO: 34 - protein, 62 aa, Ralstonia solanacearum
AIEAHMPTLRQASHSLSPERVAAIACIGGRSAVEAVRQGLPVKAIRRIRREKAPVAGPPPAS

SEQ ID NO: 35 - protein, 115 aa, Ralstonia solanacearum
SEIAKYHTTLTGQGFTHADICRISRRRQSLRVVARNYPELAAALPELTRAHIVDIARQRSGDLALQALLPVATALTAAPLRLSASQIATVAQYGERPAIQALYRLRRKLTRAPLH

SEQ ID NO: 36 - DNA, 18 bp, unidentified
  misc_feature 1..18: note = nucleic acid sequence targeted by a recombinant DNA binding protein (DBP)
  source 1..18: mol_type = other DNA
cttgggggccccttcccc

SEQ ID NO: 37 - protein, 33 aa, Legionella quateirensis
FSSQQIIRMVSHAGGANNLKAVTANHDDLQNMG

SEQ ID NO: 38 - protein, 33 aa, Legionella quateirensis
FNVEQIVRMVSHNGGSKNLKAVTDNHDDLKNMG

SEQ ID NO: 39 - protein, 33 aa, Legionella quateirensis
FNAEQIVRMVSHGGGSKNLKAVTDNHDDLKNMG

SEQ ID NO: 40 - protein, 33 aa, Legionella quateirensis
FNAEQIVSMVSNNGGSKNLKAVTDNHDDLKNMG

SEQ ID NO: 41 - protein, 33 aa, Legionella quateirensis
FNAEQIVSMVSNGGGSLNLKAVKKYHDALKDRG

SEQ ID NO: 42 - protein, 33 aa, Legionella quateirensis
FNTEQIVRMVSHDGGSLNLKAVKKYHDALRERK

SEQ ID NO: 43 - protein, 33 aa, Legionella quateirensis
FNVEQIVSIVSHGGGSLNLKAVKKYHDVLKDRE

SEQ ID NO: 44 - protein, 33 aa, Legionella quateirensis
FNAEQIVRMVSHDGGSLNLKAVTDNHDDLKNMG

SEQ ID NO: 45 - protein, 33 aa, Legionella maceachernii
FSAEQIVRIAAHDGGSRNIEAVQQAQHVLKELG

SEQ ID NO: 46 - protein, 33 aa, Legionella maceachernii
FSAEQIVSIVAHDGGSRNIEAVQQAQHILKELG

SEQ ID NO: 47 - protein, 33 aa, unidentified
  source 1..33: note = Bacterium of the order Legionellales
LDRQQILRIASHDGGSKNIAAVQKFLPKLMNFG

SEQ ID NO: 48 - protein, 33 aa, Legionella maceachernii
FSAEQIVRIAAHDGGSLNIDAVQQAQQALKELG

SEQ ID NO: 49 - protein, 33 aa, Legionella maceachernii
FSTEQIVCIAGHGGGSLNIKAVLLAQQALKDLG

SEQ ID NO: 50 - protein, 33 aa, Legionella maceachernii
YSSEQIVRVAAHGGGSLNIKAVLQAHQALKELD

SEQ ID NO: 51 - protein, 33 aa, Legionella maceachernii
FSAEQIVHIAAHGGGSLNIKAILQAHQTLKELN

SEQ ID NO: 52 - protein, 33 aa, Legionella maceachernii
FSAEQIVRIAAHIGGSRNIEAIQQAHHALKELG

SEQ ID NO: 53 - protein, 33 aa, Legionella maceachernii
FSAEQIVRIAAHIGGSHNLKAVLQAQQALKELD

SEQ ID NO: 54 - protein, 33 aa, Legionella maceachernii
FSAKHIVRIAAHIGGSLNIKAVQQAQQALKELG

SEQ ID NO: 55 - protein, 33 aa, Legionella quateirensis
FNAEQIVRMVSHKGGSKNLALVKEYFPVFSSFH

SEQ ID NO: 56 - protein, 33 aa, Legionella maceachernii
FSADQIVRIAAHKGGSHNIVAVQQAQQALKELD

SEQ ID NO: 57 - protein, 33 aa, Legionella maceachernii
FSAEQIVSIAAHVGGSHNIEAVQKAHQALKELD

SEQ ID NO: 58 - protein, 33 aa, Burkholderia sp.
FSSGETVGATVGAGGTETVAQGGTASNTTVSSG

SEQ ID NO: 59 - protein, 33 aa, Burkholderia sp.
FSGGMATSTTVGSGGTQDVLAGGAAVGGTVGTG

SEQ ID NO: 60 - protein, 33 aa, Burkholderia sp.
FSAADIVKIAGKIGGAQALQAFITHRAALIQAG

SEQ ID NO: 61 - protein, 33 aa, Burkholderia sp.
FNPTDIVKIAGNDGGAQALQAVLELEPALRERG

SEQ ID NO: 62 - protein, 33 aa, Burkholderia sp.
FNPTDIVRMAGNDGGAQALQAVFELEPAFRERS

SEQ ID NO: 63 - protein, 33 aa, Burkholderia sp.
FNPTDIVRMAGNDGGAQALQAVLELEPAFRERG

SEQ ID NO: 64 - protein, 33 aa, Burkholderia sp.
FSQVDIVKIASNDGGAQALYSVLDVEPTFRERG

SEQ ID NO: 65 - protein, 33 aa, Burkholderia sp.
FSRADIVKIAGNDGGAQALYSVLDVEPPLRERG

SEQ ID NO: 66 - protein, 33 aa, Burkholderia sp.
FSRGDIVKIAGNDGGAQALYSVLDVEPPLRERG

SEQ ID NO: 67 - protein, 33 aa, Burkholderia sp.
FNRADIVRIAGNGGGAQALYSVRDAGPTLGKRG

SEQ ID NO: 68 - protein, 33 aa, Burkholderia sp.
FRQADIVKIASNGGSAQALNAVIKLGPTLRQRG

SEQ ID NO: 69 - protein, 33 aa, Burkholderia sp.
FRQADIVKMASNGGSAQALNAVIKLGPTLRQRG

SEQ ID NO: 70 - protein, 33 aa, Burkholderia sp.
FSRADIVKIAGNGGGAQALQAVLELEPTFRERG

SEQ ID NO: 71 - protein, 33 aa, Burkholderia sp.
FSRADIVRIAGNGGGAQALYSVLDVGPTLGKRG

SEQ ID NO: 72 - protein, 33 aa, Burkholderia sp.
FSRGDIVRIAGNGGGAQALQAVLELEPTLGERG

SEQ ID NO: 73 - protein, 33 aa, Burkholderia sp.
FSRADIVKIAGNGGGAQALQAVITHRAALTQAG

SEQ ID NO: 74 - protein, 33 aa, Burkholderia sp.
FSRGDTVKIAGNIGGAQALQAVLELEPTLRERG

SEQ ID NO: 75 - protein, 33 aa, Burkholderia sp.
FNPTDIVKIAGNIGGAQALQAVLELEPAFRERG

SEQ ID NO: 76 - protein, 33 aa, Burkholderia sp.
FSAADIVKIAGNIGGAQALQAIFTHRAALIQAG

SEQ ID NO: 77 - protein, 33 aa, Burkholderia sp.
FSAADIVKIAGNIGGAQALQAVITHRATLTQAG

SEQ ID NO: 78 - protein, 33 aa, Burkholderia sp.
FSATDIVKIASNIGGAQALQAVISRRAALIQAG

SEQ ID NO: 79 - protein, 33 aa, Burkholderia sp.
FSQPDIVKIAGNIGGAQALQAVLELEPAFRERG

SEQ ID NO: 80 - protein, 33 aa, Burkholderia sp.
FSRADIVKIAGNIGGAQALQAVLELESTFRERS

SEQ ID NO: 81 - protein, 33 aa, Burkholderia sp.
FSRADIVKIAGNIGGAQALQAVLELESTLRERS

SEQ ID NO: 82 - protein, 33 aa, Burkholderia sp.
FSRGDIVKMAGNIGGAQALQAGLELEPAFRERG

SEQ ID NO: 83 - protein, 33 aa, Burkholderia sp.
FSRGDIVKMAGNIGGAQALQAVLELEPAFHERS

SEQ ID NO: 84 - protein, 33 aa, Burkholderia sp.
FTLTDIVKMAGNIGGAQALKAVLEHGPTLRQRD

SEQ ID NO: 85 - protein, 33 aa, Burkholderia sp.
FTLTDIVKMAGNIGGAQALKVVLEHGPTLRQRD

SEQ ID NO: 86 - protein, 33 aa, Burkholderia sp.
FNPTDIVKIAGNNGGAQALQAVLELEPALRERG

SEQ ID NO: 87 - protein, 33 aa, Burkholderia sp.
FNPTDIVKIAGNNGGAQALQAVLELEPALRERS

SEQ ID NO: 88 - protein, 33 aa, Burkholderia sp.
FNPTDMVKIAGNNGGAQALQAVLELEPALRERG

SEQ ID NO: 89 - protein, 33 aa, Burkholderia sp.
FSAADIVKIASNNGGAQALQALIDHWSTLSGKT

SEQ ID NO: 90 - protein, 33 aa, Burkholderia sp.
FSAADIVKIASNNGGAQALQAVISRRAALIQAG

SEQ ID NO: 91 - protein, 33 aa, Burkholderia sp.
FSAADIVKIASNNGGAQALQAVITHRAALAQAG

SEQ ID NO: 92 - protein, 33 aa, Burkholderia sp.
FSAADIVKIASNNGGARALQALIDHWSTLSGKT

SEQ ID NO: 93 - protein, 33 aa, Burkholderia sp.
FTLTDIVEMAGNNGGAQALKAVLEHGSTLDERG

SEQ ID NO: 94 - protein, 33 aa, Burkholderia sp.
FTLTDIVKMAGNNGGAQALKAVLEHGPTLDERG

SEQ ID NO: 95 - protein, 33 aa, Burkholderia sp.
FTLTDIVKMAGNNGGAQALKVVLEHGPTLRQRG

SEQ ID NO: 96 - protein, 33 aa, Burkholderia sp.
FTLTDIVKMASNNGGAQALKAVLEHGPTLDERG

SEQ ID NO: 97 - protein, 33 aa, Burkholderia sp.
FSAADIVKIAGNSGGAQALQAVISHRAALTQAG

SEQ ID NO: 98 - protein, 33 aa, Burkholderia sp.
FSGGDAVSTVVRSGGAQSVASGGTASGTTVSAG

SEQ ID NO: 99 - protein, 33 aa, Burkholderia sp.
FRQTDIVKMAGSGGSAQALNAVIKHGPTLRQRG

SEQ ID NO: 100 - protein, 33 aa, Burkholderia sp.
FSLIDIVEIASNGGAQALKAVLKYGPVLTQAGR

SEQ ID NO: 101 - protein, 33 aa, Burkholderia sp.
FSGGDAAGTVVSSGGAQNVTGGLASGTTVASGG

SEQ ID NO: 102 - protein, 33 aa, Paraburkholderia sp.
FNLTDIVEMAANSGGAQALKAVLEHGPTLRQRG

SEQ ID NO: 103 - protein, 33 aa, Paraburkholderia sp.
FNRASIVKIAGNSGGAQALQAVLKHGPTLDERG

SEQ ID NO: 104 - protein, 33 aa, Paraburkholderia sp.
FSQANIVKMAGNSGGAQALQAVLDLELVFRERG

SEQ ID NO: 105 - protein, 33 aa, Paraburkholderia sp.
FSQPDIVKMAGNSGGAQALQAVLDLELAFRERG

SEQ ID NO: 106 - protein, 33 aa, Paraburkholderia sp.
FSLIDIVEIASNGGAQALKAVLKYGPVLMQAGR

SEQ ID NO: 107 - protein, 33 aa, Francisella sp.
YKSEDIIRLASHDGGSVNLEAVLRLHSQLTRLG

SEQ ID NO: 108 - protein, 33 aa, Francisella sp.
YKPEDIIRLASHGGGSVNLEAVLRLNPQLIGLG

SEQ ID NO: 109 - protein, 33 aa, Francisella sp.
YKSEDIIRLASHGGGSVNLEAVLRLHSQLTRLG

SEQ ID NO: 110 - protein, 33 aa, Francisella sp.
YKSEDIIRLASHGGGSVNLEAVLRLNPQLIGLG

SEQ ID NO: 111 - protein, 33 aa, Legionella quateirensis
LGHKELIKIAARNGGGNNLIAVLSCYAKLKEMG

SEQ ID NO: 112 - protein, 33 aa, Paraburkholderia sp.
FNLTDIVEMAGKGGGAQALKAVLEHGPTLRQRG

SEQ ID NO: 113 - protein, 33 aa, Paraburkholderia sp.
FRQADIIKIAGNDGGAQALQAVIEHGPTLRQHG

SEQ ID NO: 114 - protein, 33 aa, Paraburkholderia sp.
FSQADIVKIAGNDGGTQALHAVLDLERMLGERG

SEQ ID NO: 115 - protein, 33 aa, Paraburkholderia sp.
FSRADIVKIAGNGGGAQALKAVLEHEATLDERG

SEQ ID NO: 116 - protein, 33 aa, Paraburkholderia sp.
FSRADIVRIAGNGGGAQALYSVLDVEPTLGKRG

SEQ ID NO: 117 - protein, 33 aa, Paraburkholderia sp.
FSQPDIVKMASNIGGAQALQAVLELEPALRERG

SEQ ID NO: 118 - protein, 33 aa, Paraburkholderia sp.
FSQPDIVKMAGNIGGAQALQAVLSLGPALRERG

SEQ ID NO: 119 - protein, 33 aa, Paraburkholderia sp.
FSQPEIVKIAGNIGGAQALHTVLELEPTLHKRG

SEQ ID NO: 120 - protein, 33 aa, Paraburkholderia sp.
FSQSDIVKIAGNIGGAQALQAVLDLESMLGKRG

SEQ ID NO: 121 - protein, 33 aa, Paraburkholderia sp.
FSQSDIVKIAGNIGGAQALQAVLELEPTLRESD

SEQ ID NO: 122 - protein, 33 aa, Paraburkholderia sp.
FNPTDIVKIAGNKGGAQALQAVLELEPALRERG

SEQ ID NO: 123 - protein, 33 aa, Paraburkholderia sp.
FSPTDIIKIAGNNGGAQALQAVLDLELMLRERG

SEQ ID NO: 124 - protein, 33 aa, Paraburkholderia sp.
FSQADIVKIAGNNGGAQALYSVLDVEPTLGKRG

SEQ ID NO: 125 - protein, 33 aa, Paraburkholderia sp.
FSRGDIVTIAGNNGGAQALQAVLELEPTLRERG

SEQ ID NO: 126 - protein, 33 aa, Paraburkholderia sp.
FSRIDIVKIAANNGGAQALHAVLDLGPTLRECG

SEQ ID NO: 127 - protein, 33 aa, Paraburkholderia sp.
FSQADIVKIVGNNGGAQALQAVFELEPTLRERG

SEQ ID NO: 128 - protein, 33 aa, Paraburkholderia sp.
FSQPDIVRITGNRGGAQALQAVLALELTLRERG

SEQ ID NO: 129 - protein, 33 aa, unidentified
  source 1..33: note = Bacterium of the order Legionellales
FKADDAVRIACRTGGSHNLKAVHKNYERLRARG

SEQ ID NO: 130 - protein, 33 aa, unidentified
  source 1..33: note = Bacterium of the order Legionellales
FNADQVIKIVGHDGGSNNIDVVQQFFPELKAFG

SEQ ID NO: 131 - protein, 33 aa, Legionella maceachernii
FSAEQIVRIAAHIGGSRNIEATIKHYAMLTQPP

SEQ ID NO: 132 - protein, 33 aa, Francisella sp.
YKSEDIIRLASHDGGSVNLEAVLRLNPQLIGLG

SEQ ID NO: 133 - protein, 33 aa, Francisella sp.
YKSEDIIRLASHDGGSINLEAVLRLNPQLIGLG

SEQ ID NO: 134 - protein, 33 aa, Francisella sp.
YKSEDIIRLASSNGGSVNLEAVLRLNPQLIGLG

SEQ ID NO: 135 - protein, 33 aa, Francisella sp.
YKSEDIIRLASSNGGSVNLEAVIAVHKALHSNG

SEQ ID NO: 136 - protein, 33 aa, unidentified
  source 1..33: note = Bacterium of the order Legionellales
FSADQVVKIAGHSGGSNNIAVMLAVFPRLRDFG

SEQ ID NO: 137 - protein, 33 aa, Francisella sp.
YKINHCVNLLKLNHDGFMLKNLIPYDSKLTGLG

SEQ ID NO: 138 - protein, 19 aa, Legionella quateirensis
  VARIANT 12: note = The amino acid at position 12 may be His, Lys, Asn, Arg, Ser, Tyr or Cys
  VARIANT 13: note = The amino acid at position 13 may be His, Lys, Gln, Asn, Ile, Gly, Asp, Val, Ala, Ser, or absent
FNAEQIVRMVSXXGGSKNL

SEQ ID NO: 139 - protein, 16 aa, Francisella sp.
  VARIANT 12: note = The amino acid at position 12 may be His, Lys, Asn, Arg, Ser, Tyr or Cys
  VARIANT 13: note = The amino acid at position 13 may be His, Lys, Gln, Asn, Ile, Gly, Asp, Val, Ala, Ser, or absent
YNKKQIVLIASXXSGG

SEQ ID NO: 140 - protein, 143 aa, Legionella quateirensis
MPDLELNFAIPLHLFDDETVFTHDATNDNSQASSSYSSKSSPASANARKRTSRKEMSGPPSKEPANTKSRRANSQNNKLSLADRLTKYNIDEEFYQTRSDSLLSLNYTKKQIERLILYKGRTSAVQQLLCKHEELLNLISPDG

SEQ ID NO: 141 - protein, 176 aa, Legionella quateirensis
ALVKEYFPVFSSFHFTADQIVALICQSKQCFRNLKKNHQQWKNKGLSAEQIVDLILQETPPKPNFNNTSSSTPSPSAPSFFQGPSTPIPTPVLDNSPAPIFSNPVCFFSSRSENNTEQYLQDSTLDLDSQLGDPTKNFNVNNFWSLFPFDDVGYHPHSNDVGYHLHSDEESPFFDF

SEQ ID NO: 142 - protein, 63 aa, Legionella quateirensis
ALVKEYFPVFSSFHFTADQIVALICQSKQCFRNLKKNHQQWKNKGLSAEQIVDLILQETPPKP

SEQ ID NO: 143 - DNA, 17 bp, synthetic construct
  source 1..17: mol_type = other DNA
tttctgtcaccaatcct

SEQ ID NO: 144 - DNA, 18 bp, synthetic construct
  source 1..18: mol_type = other DNA
tcccctccaccccacagt

SEQ ID NO: 145 - DNA, 1677 bp, synthetic construct
  source 1..1677: mol_type = other DNA
cttacgcctgaccaggtggtagcgatagccagcaacattggggggaaacaagcactcgaaactgttcagcgactgctccctgttttgtgccaagaccacggattgactcccgaccaagtggttgctatcgccagcaacggagggggtaagcaggcactggaaaccgttcaaaggctgttgccagttctctgccaggatcatggattgacaccggaccaagttgtagcaatcgccagccacgatggcggcaagcaagcactggaaacagtgcaaagattgctgcccgttctttgccaggaccacggtcttacaccagaccaagtagtggcaatcgcgagtcacgatggtggtaagcaggctcttgaaactgtacagcggctgttgcctgtgttgtgtcaagatcatggacttacgccagatcaggtggtggccatcgcgtcaaatggtgggggaaagcaagcgctcgaaacggttcagaggctcctcccggttctgtgtcaggatcatgggctgacaccggatcaagtggtagcaattgcctcacacgacggggggaaacaggcgcttgaaacggtccaacggctgctccctgtgctttgccaagatcacggcctgaccccggatcaagtagtggctattgctagcaatggtgggggtaagcaagctctggagactgtgcagagacttctccctgttctttgtcaagatcacggacttacaccggaccaggtagttgcaatcgcgagcaacggaggcgggaaacaagctctcgaaactgtacaaaggcttctcccagtactttgtcaggatcacggccttacgcccgaccaggttgtagccattgccagcaaccacggggggaagcaagccctcgaaaccgttcagaggcttctgcctgtgctttgtcaggaccacggactcacccctgatcaagtcgtggctatcgccagtaaccacgggggaaaacaagcccttgaaacggtgcaaagacttcttccggtgctgtgtcaggaccatgggcttacgccagaccaggtggtggcgattgccagtaatcatggcggtaagcaggcgctcgaaactgtgcagcggctgctgccggttctttgccaagaccatggacttacccccgatcaagtggttgccatcgcgagtaatcacggcggcaaacaggcgctggaaacggtacaacggctgttgccggtcctttgccaggatcacgggcttacgcctgatcaagttgttgcgatcgccagcaatcacgggggcaagcaagctcttgaaacggttcaaagactgctcccggttttgtgtcaagaccatggtttgacccctgaccaagttgttgcaattgccagccacgacggtggtaaacaggctctcgaaacagtccaaaggcttttgccggtactctgtcaagaccacggccttactccggaccaggtggttgccattgcgagtcacgacgggggcaaacaggcactcgaaacggtccagagacttttgcctgtgctctgccaagatcatggtctgactcctgaccaagtggtggcaatcgcctcacacgatggtgggaagcaggccctcgaaacggtacagcgactgttgcccgtattgtgccaggaccatggcctgacgccggaccaggttgtggccatagctagccacgatggagga

SEQ ID NO: 146 - DNA, 1881 bp, synthetic construct
  source 1..1881: mol_type = other DNA
cttacccccgatcaagtcgtggctatcgctagtaacattggaggtaaacaggcccttgaaacagttcagagacttttgccagtactttgccaggatcatggcttgacaccagaccaggtcgtcgcaatagcttctaacggtgggggtaagcaggctctggaaacagtgcagaggctcctccccgtgttgtgtcaggaccacgggttgaccccggatcaggtggtcgcgattgccagtcacgatggtggaaaacaagcactcgagactgttcagcgcttgcttcctgttttgtgccaggatcatgggcttacacccgatcaggtagttgctatcgcgtcccacgatggaggtaagcaggcccttgagactgtgcaacggctgttgcctgtactctgtcaagaccacggtcttactccagatcaggtcgttgcaatcgcgagtaacggtggtggcaaacaagccctggaaaccgtgcagcgcctcctccccgtgctttgtcaagatcacggcctgacacccgatcaagtagttgccatcgcgtctcacgatggagggaagcaggctcttgaaacggtgcaacgcttgctgccggtcttgtgtcaggaccatggcctgacccctgaccaagtcgtagctatcgcttcaaacggtggagggaaacaagcccttgagacagtccagcggctcctgccagtgctctgccaagatcatggcctcacccctgatcaggtcgtggccatcgcaagcaacggtggtggtaaacaggctctggagacagtccaacggctcttgccagttctctgccaggaccatgggcttactccggaccaggtggttgccatcgcctcaaaccatggggggaaacaggcattggagacagtgcagagactcctgcccgtgttgtgccaggatcacggacttacgcctgaccaggtagtggcaattgcctccaaccatggcggaaaacaggctttggagactgtccagagactgttgccagttctctgtcaggaccacggtctgaccccagatcaagttgtcgcaatcgcaagtaaccatggggggaagcaagccctcgaaactgtgcagcgcctgctgccagtcctgtgccaggaccacggattgacaccagatcaggtggtagccattgcaagtaaccatggcgggaaacaagccctcgaaacggtgcaaagactccttcccgtgctgtgtcaggatcatggccttacccctgatcaggtggttgctatcgcctctaaccatggcggtaagcaggcactcgaaacagttcagcggcttctgcctgtcttgtgtcaagaccatggcctcactccagaccaggtcgtagcaattgccagccacgatgggggaaagcaagcgctcgagactgtgcagcggctgctcccagtgctttgtcaggaccatggactgacacctgatcaggttgttgcaattgcatctcacgatggtgggaagcaagcgttggaaaccgtccagcgcctgctccccgttctctgccaggatcatggattgactcccgaccaagttgtggccatcgcctcccacgatggaggcaagcaggcacttgaaactgttcagcggctgttgcccgttctttgtcaggatcacggccttactccggatcaagtggtagctatcgcatcccacgatgggggcaaacaagctctcgaaacagtgcagcgcttgctgcccgtgctctgtcaagatcatggtctgacacccgaccaggtggtggccatagcgagcaacggtggcggcaagcaggccctggaaacggtgcagaggctgctccctgtcctgtgccaagaccacggcctcacaccggatcaggtcgtggctatagctagcaacggtggagga

SEQ ID NO: 147 - DNA, 1677 bp, synthetic construct
  source 1..1677: mol_type = other DNA
cttaccccggaccaggtggttgctatcgcctccaacggtggaggcaagcaggctctcgaaactgtgcagcggctcctccccgtgctctgtcaggaccatggcttgacacccgatcaagtagtcgctatcgcctcaaaccatggtggcaagcaggccttggagacagtgcaacgactgctgccagttctgtgtcaggaccacgggctgaccccagaccaggtcgtcgccatagcgtcacacgatggaggtaaacaagcactggagactgtccagaggttgctcccagtcctgtgccaggaccatggattgactcccgaccaggttgttgccattgcatccaacggtggtgggaaacaggctcttgagactgtccaaagactgttgccggtgctgtgccaagaccacggtcttactccggatcaggtcgttgcgatagcaagtaacggtggggggaaacaggccctggaaactgtgcagaggctgctgcccgttctctgtcaagatcacgggctgacaccagatcaggtagttgccatcgcaagcaacggtgggggcaagcaggcgctcgaaacggtgcaacggctgctgcctgtcctctgccaagaccatggcctgaccccggatcaggtagtggctatcgcttctaacggtggaggcaaacaggcactggaaacagtccagcggttgctgcccgtgctttgccaagatcatggcttgacgcctgaccaagtcgtggcaattgcttccaacattggcggaaagcaggccttggaaaccgtgcagcgactcctccctgtgctctgccaggaccatggccttactcccgatcaggtcgtggccattgcctcaaacggtggcggcaagcaggcacttgagacagttcagcgcctgctgcctgttttgtgccaggatcacgggttgacccctgaccaggttgtggcaatagcctctcacgatggtggtaagcaagccctcgagacagtgcagcgcctgttgcctgtgctttgccaagaccacggattgacgcccgatcaggtggttgccatagccagcaacattggagggaagcaggccctggagacagtgcagcggctgcttcctgtcttgtgccaagatcacggcctcacccccgatcaggtagtcgcaatcgcatctcacgatggaggaaagcaggccctcgaaacggtgcagaggcttctgcccgtgttgtgccaggatcatggccttacccctgatcaggtcgtcgctatcgcgtccaacattgggggtaaacaggctctcgagacagttcaaagactccttcctgttctgtgtcaagatcatggcctgacacctgatcaagtggtcgcaatagcttcaaaccatggtggaaagcaggcactcgaaacagtccaacggcttctgcccgtactctgtcaggaccacggactgacacctgatcaggttgtggcgattgcgagtaaccatggaggtaagcaggcacttgaaactgtccagagactccttccggtcctttgccaggatcacggtctgacgcctgatcaggtggtggctatagctagtcacgatggcgggaagcaggcattggagacagtacagcggctgttgcccgtattgtgtcaagaccacggcctgactccggaccaagtggtggctatagctagcaacggtggagga

SEQ ID NO: 148 - protein, 703 aa, synthetic construct
MDYKDHDGDYKDHDIDYKDDDDKMAPKKKRKVGIHRGVPMVDLRTLGYSQQQQEKIKPKVRSTVAQHHEALVGHGFTHAHIVALSQHPAALGTVAVKYQDMIAALPEATHEAIVGVGKQWSGARALEALLTVAGELRGPPLQLDTGQLLKIAKRGGVTAVEAVHAWRNALTGAPLNLTPDQVVAIASNIGGKQALETVQRLLPVLCQDHGLTPDQVVAIASNGGGKQALETVQRLLPVLCQDHGLTPDQVVAIASHDGGKQALETVQRLLPVLCQDHGLTPDQVVAIASHDGGKQALETVQRLLPVLCQDHGLTPDQVVAIASNGGGKQALETVQRLLPVLCQDHGLTPDQVVAIASHDGGKQALETVQRLLPVLCQDHGLTPDQVVAIASNGGGKQALETVQRLLPVLCQDHGLTPDQVVAIASNGGGKQALETVQRLLPVLCQDHGLTPDQVVAIASNHGGKQALETVQRLLPVLCQDHGLTPDQVVAIASNHGGKQALETVQRLLPVLCQDHGLTPDQVVAIASNHGGKQALETVQRLLPVLCQDHGLTPDQVVAIASNHGGKQALETVQRLLPVLCQDHGLTPDQVVAIASNHGGKQALETVQRLLPVLCQDHGLTPDQVVAIASHDGGRPALESIVAQLSRPDPALAALTNDHLVALACLGGRPALDAVKKGLPHAPALIKRTNRRIPERTSHRVAGS

SEQ ID NO: 149 - protein, 771 aa, synthetic construct
MDYKDHDGDYKDHDIDYKDDDDKMAPKKKRKVGIHRGVPMVDLRTLGYSQQQQEKIKPKVRSTVAQHHEALVGHGFTHAHIVALSQHPAALGTVAVKYQDMIAALPEATHEAIVGVGKQWSGARALEALLTVAGELRGPPLQLDTGQLLKIAKRGGVTAVEAVHAWRNALTGAPLNLTPDQVVAIASHDGGKQALETVQRLLPVLCQDHGLTPDQVVAIASHDGGKQALETVQRLLPVLCQDHGLTPDQVVAIASNGGGKQALETVQRLLPVLCQDHGLTPDQVVAIASHDGGKQALETVQRLLPVLCQDHGLTPDQVVAIASNGGGKQALETVQRLLPVLCQDHGLTPDQVVAIASNGGGKQALETVQRLLPVLCQDHGLTPDQVVAIASNHGGKQALETVQRLLPVLCQDHGLTPDQVVAIASNHGGKQALETVQRLLPVLCQDHGLTPDQVVAIASNHGGKQALETVQRLLPVLCQDHGLTPDQVVAIASNHGGKQALETVQRLLPVLCQDHGLTPDQVVAIASNHGGKQALETVQRLLPVLCQDHGLTPDQVVAIASHDGGKQALETVQRLLPVLCQDHGLTPDQVVAIASHDGGKQALETVQRLLPVLCQDHGLTPDQVVAIASNGGGKQALETVQRLLPVLCQDHGLTPDQVVAIASNGGGKQALETVQRLLPVLCQDHGLTPDQVVAIASHDGGRPALESIVAQLSRPDPALAALTNDHLVALACLGGRPALDAVKKGLPHAPALIKRTNRRIPERTSHRVAGS

SEQ ID NO: 150 - protein, 134 aa, synthetic construct
MVDLRTLGYSQQQQEKIKPKVRSTVAQHHEALVGHGFTHAHIVALSQHPAALGTVAVKYQDMIAALPEATHEAIVGVGKQWSGARALEALLTVAGELRGPPLQLDTGQLLKIAKRGGVTAVEAVHAWRNALTGA

SEQ ID NO: 151 - protein, 63 aa, synthetic construct
SIVAQLSRPDPALAALTNDHLVALACLGGRPALDAVKKGLPHAPALIKRTNRRIPERTSHRVA

SEQ ID NO: 152 - protein, 20 aa, synthetic construct
LTPDQVVAIASNIGGRPALE

SEQ ID NO: 153 - protein, 20 aa, synthetic construct
LTPDQVVAIASNGGGRPALE

SEQ ID NO: 154 - protein, 20 aa, synthetic construct
LTPDQVVAIASHDGGRPALE

SEQ ID NO: 155 - protein, 20 aa, synthetic construct
LTPDQVVAIASNHGGRPALE

SEQ ID NO: 156 - protein, 805 aa, synthetic construct
MDYKDHDGDYKDHDIDYKDDDDKMAPKKKRKVGIHRGVPMVDLRTLGYSQQQQEKIKPKVRSTVAQHHEALVGHGFTHAHIVALSQHPAALGTVAVKYQDMIAALPEATHEAIVGVGKQWSGARALEALLTVAGELRGPPLQLDTGQLLKIAKRGGVTAVEAVHAWRNALTGAPLNLTPDQVVAIASNIGGKQALETVQRLLPVLCQDHGLTPDQVVAIASNGGGKQALETVQRLLPVLCQDHGLTPDQVVAIASHDGGKQALETVQRLLPVLCQDHGLTPDQVVAIASHDGGKQALETVQRLLPVLCQDHGLTPDQVVAIASNGGGKQALETVQRLLPVLCQDHGLTPDQVVAIASHDGGKQALETVQRLLPVLCQDHGLTPDQVVAIASNGGGKQALETVQRLLPVLCQDHGLTPDQVVAIASNGGGKQALETVQRLLPVLCQDHGLTPDQVVAIASNHGGKQALETVQRLLPVLCQDHGLTPDQVVAIASNHGGKQALETVQRLLPVLCQDHGLTPDQVVAIASNHGGKQALETVQRLLPVLCQDHGLTPDQVVAIASNHGGKQALETVQRLLPVLCQDHGLTPDQVVAIASNHGGKQALETVQRLLPVLCQDHGLTPDQVVAIASHDGGKQALETVQRLLPVLCQDHGLTPDQVVAIASHDGGKQALETVQRLLPVLCQDHGLTPDQVVAIASHDGGKQALETVQRLLPVLCQDHGLTPDQVVAIASHDGGRPALESIVAQLSRPDPALAALTNDHLVALACLGGRPALDAVKKGLPHAPALIKRTNRRIPERTSHRVAGS

SEQ ID NO: 157 - protein, 907 aa, synthetic construct
MDYKDHDGDYKDHDIDYKDDDDKMAPKKKRKVGIHRGVPMVDLRTLGYSQQQQEKIKPKVRSTVAQHHEALVGHGFTHAHIVALSQHPAALGTVAVKYQDMIAALPEATHEAIVGVGKQWSGARALEALLTVAGELRGPPLQLDTGQLLKIAKRGGVTAVEAVHAWRNALTGAPLNLTPDQVVAIASHDGGKQALETVQRLLPVLCQDHGLTPDQVVAIASHDGGKQALETVQRLLPVLCQDHGLTPDQVVAIASNGGGKQALETVQRLLPVLCQDHGLTPDQVVAIASHDGGKQALETVQRLLPVLCQDHGLTPDQVVAIASNGGGKQALETVQRLLPVLCQDHGLTPDQVVAIASNGGGKQALETVQRLLPVLCQDHGLTPDQVVAIASNHGGKQALETVQRLLPVLCQDHGLTPDQVVAIASNHGGKQALETVQRLLPVLCQDHGLTPDQVVAIASNHGGKQALETVQRLLPVLCQDHGLTPDQVVAIASNHGGKQALETVQRLLPVLCQDHGLTPDQVVAIASNHGGKQALETVQRLLPVLCQDHGLTPDQVVAIASHDGGKQALETVQRLLPVLCQDHGLTPDQVVAIASHDGGKQALETVQRLLPVLCQDHGLTPDQVVAIASHDGGKQALETVQRLLPVLCQDHGLTPDQVVAIASHDGGKQALETVQRLLPVLCQDHGLTPDQVVAIASNGGGKQALETVQRLLPVLCQDHGLTPDQVVAIASNGGGKQALETVQRLLPVLCQDHGLTPDQVVAIASHDGGKQALETVQRLLPVLCQDHGLTPDQVVAIASHDGGKQALETVQRLLPVLCQDHGLTPDQVVAIASHDGGRPALESIVAQLSRPDPALAALTNDHLVALACLGGRPALDAVKKGLPHAPALIKRTNRRIPERTSHRVAGS

SEQ ID NO: 158 - DNA, 24 bp, unidentified
  misc_feature 1..24: note = target sequence for gamma-globin proximal promoter
  source 1..24: mol_type = other DNA
tatcctcttgggggccccttcccc

SEQ ID NO: 159 - DNA, 23 bp, unidentified
  misc_feature 1..23: note = target sequence for gamma-globin proximal promoter
  source 1..23: mol_type = other DNA
tatcctcttgggggccccttccc

SEQ ID NO: 160 - DNA, 22 bp, unidentified
  misc_feature 1..22: note = target sequence for gamma-globin proximal promoter
  source 1..22: mol_type = other DNA
tatcctcttgggggccccttcc

SEQ ID NO: 161 - DNA, 21 bp, unidentified
  misc_feature 1..21: note = target sequence for gamma-globin proximal promoter
  source 1..21: mol_type = other DNA
tatcctcttgggggccccttc

SEQ ID NO: 162 - DNA, 20 bp, unidentified
  misc_feature 1..20: note = target sequence for gamma-globin proximal promoter
  source 1..20: mol_type = other DNA
tatcctcttgggggcccctt

SEQ ID NO: 163 - DNA, 19 bp, unidentified
  misc_feature 1..19: note = target sequence for gamma-globin proximal promoter
  source 1..19: mol_type = other DNA
tatcctcttgggggcccct

SEQ ID NO: 164 - DNA, 18 bp, unidentified
  misc_feature 1..18: note = target sequence for gamma-globin proximal promoter
  source 1..18: mol_type = other DNA
tatcctcttgggggcccc

SEQ ID NO: 165 - DNA, 17 bp, unidentified
  misc_feature 1..17: note = target sequence for gamma-globin proximal promoter
  source 1..17: mol_type = other DNA
tatcctcttgggggccc

SEQ ID NO: 166 - DNA, 16 bp, unidentified
  misc_feature 1..16: note = target sequence for gamma-globin proximal promoter
  source 1..16: mol_type = other DNA
tatcctcttgggggcc

SEQ ID NO: 167 - DNA, 15 bp, unidentified
  misc_feature 1..15: note = target sequence for gamma-globin proximal promoter
  source 1..15: mol_type = other DNA
tatcctcttgggggc

SEQ ID NO: 168 - DNA, 24 bp, unidentified
  misc_feature 1..24: note = target sequence for gamma-globin proximal promoter
  source 1..24: mol_type = other DNA
tcctcttgggggccccttccccac

SEQ ID NO: 169 - DNA, 23 bp, unidentified
  misc_feature 1..23: note = target sequence for gamma-globin proximal promoter
  source 1..23: mol_type = other DNA
tcctcttgggggccccttcccca

SEQ ID NO: 170 - DNA, 22 bp, unidentified
  misc_feature 1..22: note = target sequence for gamma-globin proximal promoter
  source 1..22: mol_type = other DNA
tcctcttgggggccccttcccc

SEQ ID NO: 171 - DNA, 21 bp, unidentified
  misc_feature 1..21: note = target sequence for gamma-globin proximal promoter
  source 1..21: mol_type = other DNA
tcctcttgggggccccttccc

SEQ ID NO: 172 - DNA, 20 bp, unidentified
  misc_feature 1..20: note = target sequence for gamma-globin proximal promoter
  source 1..20: mol_type = other DNA
tcctcttgggggccccttcc

SEQ ID NO: 173 - DNA, 19 bp, unidentified
  misc_feature 1..19: note = target sequence for gamma-globin proximal promoter
  source 1..19: mol_type = other DNA
tcctcttgggggccccttc

SEQ ID NO: 174 - DNA, 18 bp, unidentified
  misc_feature 1..18: note = target sequence for gamma-globin proximal promoter
  source 1..18: mol_type = other DNA
tcctcttgggggcccctt

SEQ ID NO: 175 - DNA, 17 bp, unidentified
  misc_feature 1..17: note = target sequence for gamma-globin proximal promoter
  source 1..17: mol_type = other DNA
tcctcttgggggcccct

SEQ ID NO: 176 - DNA, 16 bp, unidentified
  misc_feature 1..16: note = target sequence for gamma-globin proximal promoter
  source 1..16: mol_type = other DNA
tcctcttgggggcccc

SEQ ID NO: 177 - DNA, 15 bp, unidentified
  misc_feature 1..15: note = target sequence for gamma-globin proximal promoter
  source 1..15: mol_type = other DNA
tcctcttgggggccc

SEQ ID NO: 178 - DNA, 19 bp, unidentified
  misc_feature 1..19: note = target sequence for gamma-globin proximal promoter
  source 1..19: mol_type = other DNA
tcaccctgtggagccacac

SEQ ID NO: 179 - DNA, 18 bp, unidentified
  misc_feature 1..18: note = target sequence for gamma-globin proximal promoter
  source 1..18: mol_type = other DNA
ttgcttttatcacaggct

SEQ ID NO: 180 - DNA, 17 bp, unidentified
  misc_feature 1..17: note = nucleic acid sequence targeted by a recombinant DNA binding protein (DBP)
  source 1..17: mol_type = other DNA
tgcttttatcacaggct

SEQ ID NO: 181 - DNA, 18 bp, unidentified
  misc_feature 1..18: note = nucleic acid sequence targeted by a recombinant DNA binding protein (DBP)
  source 1..18: mol_type = other DNA
caccctgtggagccacac

SEQ ID NO: 182 - DNA, 23 bp, unidentified
  misc_feature 1..23: note = nucleic acid sequence targeted by a recombinant DNA binding protein (DBP)
  source 1..23: mol_type = other DNA
cctcttgggggccccttccccac

SEQ ID NO: 183 - DNA, 22 bp, unidentified
  misc_feature 1..22: note = nucleic acid sequence targeted by a recombinant DNA binding protein (DBP)
  source 1..22: mol_type = other DNA
cctcttgggggccccttcccca

SEQ ID NO: 184 - DNA, 21 bp, unidentified
  misc_feature 1..21: note = nucleic acid sequence targeted by a recombinant DNA binding protein (DBP)
  source 1..21: mol_type = other DNA
cctcttgggggccccttcccc

SEQ ID NO: 185 - DNA, 19 bp, unidentified
  misc_feature 1..19: note = nucleic acid sequence targeted by a recombinant DNA binding protein (DBP)
  source 1..19: mol_type = other DNA
cctcttgggggccccttcc

SEQ ID NO: 186 - DNA, 18 bp, unidentified
  misc_feature 1..18: note = nucleic acid sequence targeted by a recombinant DNA binding protein (DBP)
  source 1..18: mol_type = other DNA
cctcttgggggccccttc

SEQ ID NO: 187 - DNA, 16 bp, unidentified
  misc_feature 1..16: note = nucleic acid sequence targeted by a recombinant DNA binding protein (DBP)
  source 1..16: mol_type = other DNA
cctcttgggggcccct

SEQ ID NO: 188 - DNA, 15 bp, unidentified
  misc_feature 1..15: note = nucleic acid sequence targeted by a recombinant DNA binding protein (DBP)
  source 1..15: mol_type = other DNA
cctcttgggggcccc

SEQ ID NO: 189 - DNA, 14 bp, unidentified
  misc_feature 1..14: note = nucleic acid sequence targeted by a recombinant DNA binding protein (DBP)
  source 1..14: mol_type = other DNA
cctcttgggggccc

SEQ ID NO: 190 - DNA, 13 bp, unidentified
  misc_feature 1..13: note = nucleic acid sequence targeted by a recombinant DNA binding protein (DBP)
  source 1..13: mol_type = other DNA
cctcttgggggcc

SEQ ID NO: 191 - DNA, 16 bp, unidentified
  misc_feature 1..16: note = nucleic acid sequence targeted by a recombinant DNA binding protein (DBP)
  source 1..16: mol_type = other DNA
atcctcttgggggccc

SEQ ID NO: 192 - DNA, 18 bp, unidentified
  misc_feature 1..18: note = nucleic acid sequence targeted by a recombinant DNA binding protein (DBP)
  source 1..18: mol_type = other DNA
atcctcttgggggcccct

SEQ ID NO: 193 - DNA, 19 bp, unidentified
  misc_feature 1..19: note = nucleic acid sequence targeted by a recombinant DNA binding protein (DBP)
  source 1..19: mol_type = other DNA
atcctcttgggggcccctt

SEQ ID NO: 194 - DNA, 20 bp, unidentified
  misc_feature 1..20: note = nucleic acid sequence targeted by a recombinant DNA binding protein (DBP)
  source 1..20: mol_type = other DNA
atcctcttgggggccccttc

SEQ ID NO: 195 - DNA, 21 bp, unidentified
  misc_feature 1..21: note = nucleic acid sequence targeted by a recombinant DNA binding protein (DBP)
  source 1..21: mol_type = other DNA
atcctcttgggggccccttcc

SEQ ID NO: 196 - DNA, 22 bp, unidentified
  misc_feature 1..22: note = nucleic acid sequence targeted by a recombinant DNA binding protein (DBP)
  source 1..22: mol_type = other DNA
atcctcttgggggccccttccc

SEQ ID NO: 197 - DNA, 23 bp, unidentified
  misc_feature 1..23: note = nucleic acid sequence targeted by a recombinant DNA binding protein (DBP)
  source 1..23: mol_type = other DNA
atcctcttgggggccccttcccc

SEQ ID NO: 198 - DNA, 15 bp, unidentified
  misc_feature 1..15: note = nucleic acid sequence targeted by a recombinant DNA binding protein (DBP)
  source 1..15: mol_type = other DNA
atcctcttgggggcc

SEQ ID NO: 199 - DNA, 14 bp, unidentified
  misc_feature 1..14: note = nucleic acid sequence targeted by a recombinant DNA binding protein (DBP)
  source 1..14: mol_type = other DNA
atcctcttgggggc

SEQ ID NO: 200 - DNA, 13 bp, unidentified
  misc_feature 1..13: note = nucleic acid sequence targeted by a recombinant DNA binding protein (DBP)
  source 1..13: mol_type = other DNA
tcctcttgggggc

SEQ ID NO: 201 - DNA, 12 bp, unidentified
  misc_feature 1..12: note = nucleic acid sequence targeted by a recombinant DNA binding protein (DBP)
  source 1..12: mol_type = other DNA
cctcttgggggc

SEQ ID NO: 202 - DNA, 20 bp, synthetic construct
  source 1..20: mol_type = other DNA
tcttgggggccccttcccca

SEQ ID NO: 203 - DNA, 19 bp, synthetic construct
  source 1..19: mol_type = other DNA
tcttgggggccccttcccc

SEQ ID NO: 204 - DNA, 18 bp, synthetic construct
  source 1..18: mol_type = other DNA
tcttgggggccccttccc

SEQ ID NO: 205 - DNA, 17 bp, synthetic construct
  source 1..17: mol_type = other DNA
tcttgggggccccttcc

SEQ ID NO: 206 - DNA, 16 bp, synthetic construct
  source 1..16: mol_type = other DNA
tcttgggggccccttc

SEQ ID NO: 207 - DNA, 15 bp, synthetic construct
  source 1..15: mol_type = other DNA
tcttgggggcccctt

SEQ ID NO: 208 - DNA, 20 bp, synthetic construct
  source 1..20: mol_type = other DNA
ttaagcagcagtatcctctt

SEQ ID NO: 209 - DNA, 17 bp, synthetic construct
  source 1..17: mol_type = other DNA
tagcagtatcctcttgg

SEQ ID NO: 210 - DNA, 19 bp, synthetic construct
  source 1..19: mol_type = other DNA
tagcagtatcctcttgggg

SEQ ID NO: 211 - DNA, 17 bp, synthetic construct
  source 1..17: mol_type = other DNA
cctcttgggggcccctt

SEQ ID NO: 212 - DNA, 48 bp, synthetic construct
  source 1..48: mol_type = other DNA
aaacccttcctggagcctgtgataaaagcaactgttagcttgcactag

SEQ ID NO: 213 - DNA, 48 bp, synthetic construct
  source 1..48: mol_type = other DNA
ctagtgcaagctaacagttgcttttatcacaggctccaggaagggttt

SEQ ID NO: 214 - DNA, 37 bp, synthetic construct
  source 1..37: mol_type = other DNA
gatagtgtggggaaggggcccccaagaggatactgct

SEQ ID NO: 215 - DNA, 17 bp, unidentified
  misc_feature 1..17: note = nucleic acid sequence targeted by a recombinant DNA binding protein (DBP)
  source 1..17: mol_type = other DNA
cttgggggccccttccc

SEQ ID NO: 216 - DNA, 16 bp, unidentified
  misc_feature 1..16: note = nucleic acid sequence targeted by a recombinant DNA binding protein (DBP)
  source 1..16: mol_type = other DNA
cttgggggccccttcc

SEQ ID NO: 217 - DNA, 15 bp, unidentified
  misc_feature 1..15: note = nucleic acid sequence targeted by a recombinant DNA binding protein (DBP)
  source 1..15: mol_type = other DNA
cttgggggccccttc

SEQ ID NO: 218 - DNA, 14 bp, unidentified
  misc_feature 1..14: note = nucleic acid sequence targeted by a recombinant DNA binding protein (DBP)
  source 1..14: mol_type = other DNA
cttgggggcccctt

SEQ ID NO: 219 - DNA, 19 bp, unidentified
  misc_feature 1..19: note = nucleic acid sequence targeted by a recombinant DNA binding protein (DBP)
  source 1..19: mol_type = other DNA
taagcagcagtatcctctt

SEQ ID NO: 220 - DNA, 16 bp, unidentified
  misc_feature 1..16: note = nucleic acid sequence targeted by a recombinant DNA binding protein (DBP)
  source 1..16: mol_type = other DNA
agcagtatcctcttgg

SEQ ID NO: 221 - DNA, 18 bp, unidentified
  misc_feature 1..18: note = nucleic acid sequence targeted by a recombinant DNA binding protein (DBP)
  source 1..18: mol_type = other DNA
agcagtatcctcttgggg